European Patent Specification EP 4 139 448 B1, published April 1, 2026. Title: A MODIFIED BACTERIAL HYALURONIDASE POLYPEPTIDE, PRODUCTION PROCESS, PHARMACEUTICAL COMPOSITIONS AND THEIR USES. Applicant: PharmACT Holding AG. The sequence listing filed with the application follows.

SEQUENCE LISTING (8 sequences)

SEQ ID NO: 1 - protein, 740 aa, Streptococcus pneumoniae
  Modified bacterial hyaluronidase D016
MGWSHPQFEKASVKDTYTDRLDDWNGIIAGNQYYDSKNDQMAKLNQELEGKVADSLSSISSQADRIYLWEKFSNYKTSANLTATYRKLEEMAKQVTNPSSRYYQDETVVRTVRDSMEWMHKHVYNSEKSIVGNWWDYEIGTPRAINNTLSLMKEYFSDEEIKKYTDVIEKFVPDPEHFRKTTDNPFKALGGNLVDMGRVKVIAGLLRKDDQEISSTIRSIEQVFKLVDQGEGFYQDGSYIDHTNVAYTGAYGNVLIDGLSQLLPVIQKTKNPIDKDKMQTMYHWIDKSFAPLLVNGELMDMSRGRSISRANSEGHVAAVEVLRGIHRIADMSEGETKQRLQSLVKTIVQSDSYYDVFKNLKTYKDISLMQSLLSDAGVASVPRTSYLSAFNKMDKTAMYNAEKGFGFGLSLFSSRTLNYEHMNKENKRGWYTSDGMFYLYNGDLSHYSDGYWPTVNPYKMPGTTETDAKRADSDTGKVLPSAFVGTSKLDDANATATMDFTNWNQTLTAHKSWFMLKDKIAFLGSNIQNTSTDTAATTIDQRKLESSNPYKVYVNDKEASLTEQEKDYPETQSGFLESSDSKKNIGYFFFKKSSISMSKALQKGAWKDINEGQSDKEVENEFLTISQAHKQNGDSYGYMLIPNVDRATFNQMIKELESSLIENNETLQSVYDAKQGVWGIVKYDDSVSTISNQFQVLKRGVYTIRKEGDEYKIAYYNPETQESAPDQEVFKKLEHHHHHH

SEQ ID NO: 2 - DNA, 2251 bp, Streptococcus pneumoniae
  DNA Sequence encoding modified bacterial hyaluronidase D016
ccatgggctggagccatccgcagtttgaaaaagcaagcgtgaaggatacgtacacggaccgcttagatgactggaacgggatcatcgcggggaaccagtactatgatagcaaaaacgaccaaatggcaaaattaaatcaagaattagaaggtaaggtcgcggattcactctcaagcattagcagccaagctgaccggatctatttatgggaaaaatttagcaactataaaacaagcgccaaccttacggcaacgtatcgaaaattagaggagatggcaaagcaggtaacgaacccgagcagccgctattatcaggatgaaacggtcgtgcggacggtccgagattcaatggaatggatgcataaacatgtctacaacagcgaaaagtcaattgtggggaattggtgggattatgaaatcggcacgccgcgcgcaatcaataacacgttaagccttatgaaagaatacttcagcgatgaggaaattaaaaaatatacggatgtaattgaaaaatttgtcccagatccagaacatttccggaagacaacggataatccgttcaaggcgctcggcggtaatttagtggatatgggtcgagtcaaagtcatagcgggcttacttcgcaaggatgatcaggaaattagcagcacgattcggtcaattgagcaggtattcaagttagtcgaccagggcgaaggcttttatcaggatggttcatatatcgaccacacgaacgtggcatatacaggcgcgtatgggaacgtgttaattgatgggttgagccagcttttaccggtcattcagaagacgaagaacccgatcgataaagataaaatgcagacgatgtaccactggattgataaatcatttgcgccgttacttgtaaacggtgagcttatggatatgagccgcggtcggtcaatcagccgcgccaactcagaggggcacgtagcagccgtcgaagtcctccgggggattcaccggatagctgatatgagcgaaggtgaaacgaaacagcgcttacaaagcttagtaaagacgattgtgcagtcagatagctattatgatgtctttaagaacttaaagacgtataaggatatcagcttaatgcagtcattattaagcgatgccggtgtcgccagcgtgccgcggacgagctacctcagcgcatttaataagatggataaaacggcaatgtacaacgccgagaaagggtttggttttgggttaagcttgttttcaagccgcacgttaaactacgaacacatgaataaggaaaacaaacgcggctggtatacaagcgatgggatgttctatttatacaacggggatttaagccactattcagatgggtactggccgacggtgaacccgtataagatgccgggcacgacggagacagatgcgaagcgggctgattcagatacgggcaaagtgttacccagcgcgttcgtgggtacatcaaaactcgatgatgcaaacgctacggccacgatggatttcacgaattggaaccagacgttaacggcgcataagtcatggtttatgctcaaggataagattgcatttttaggttcaaacatccagaatacgagcacggatacggcggccacgacgattgaccaacggaaacttgaaagcagcaacccgtataaagtctatgtcaacgataaagaagcatcattaacggaacaggaaaaggattatccggaaacgcagagcgggtttttagaatcatcagattcaaaaaagaacattggctactttttctttaagaagagcagcatcagcatgagcaaggcgttacagaagggtgcatggaaggatatcaacgaaggtcaaagcgacaaggaagtggaaaacgaatttttaacaattagccaagcgcataagcagaacggtgatagctatgggtatatgttgattccgaatgtagatcgcgcaacgttcaaccagatgataaaagagttagaatcatcattgatcgaaaacaatgaaacgttacaaagcgtgtatgatgcaaaacagggtgtgtgggggattgtaaaatatgatgatagcgtcagcacgatttcaaatcagttccaggtgttaaaacgcggtgtctatacgattcggaaagaaggggatgaatataagattgcatactataacccggaaacgcaagaaagcgcgccggatcaagaagtctttaaaaagctcgagcatcatcatcatcatcactaaccactcgacttcttttggagctgagc

SEQ ID NO: 3 - protein, 949 aa, Streptococcus pneumoniae
  Wild Type bacterial hyaluronidase sequence
MVPIEAKKKYKLRFKIKTDNKVGIAKVRIIEESGKDKRLWNSATTSGTKDWQTIEADYSPTLDVDKIKLELFYETGTGTVSFKDIELVEVADQPSEDSQTDKQLEEKIDLPIGKKHVFPLADYTYKVENPDVASVKNGILEPLKEGTTNVIVSKDGKEVKKIPLKILASVKDTYTDRLDDWNGIIAGNQYYDSKNDQMAKLNQELEGKVADSLSSISSQADRIYLWEKFSNYKTSANLTATYRKLEEMAKQVTNPSSRYYQDETVVRTVRDSMEWMHKHVYNSEKSIVGNWWDYEIGTPRAINNTLSLMKEYFSDEEIKKYTDVIEKFVPDPEHFRKTTDNPFKALGGNLVDMGRVKVIAGLLRKDDQEISSTIRSIEQVFKLVDQGEGFYQDGSYIDHTNVAYTGAYGNVLIDGLSQLLPVIQKTKNPIDKDKMQTMYHWIDKSFAPLLVNGELMDMSRGRSISRANSEGHVAAVEVLRGIHRIADMSEGETKQRLQSLVKTIVQSDSYYDVFKNLKTYKDISLMQSLLSDAGVASVPRTSYLSAFNKMDKTAMYNAEKGFGFGLSLFSSRTLNYEHMNKENKRGWYTSDGMFYLYNGDLSHYSDGYWPTVNPYKMPGTTETDAKRADSDTGKVLPSAFVGTSKLDDANATATMDFTNWNQTLTAHKSWFMLKDKIAFLGSNIQNTSTDTAATTIDQRKLESSNPYKVYVNDKEASLTEQEKDYPETQSGFLESSDSKKNIGYFFFKKSSISMSKALQKGAWKDINEGQSDKEVENEFLTISQAHKQNGDSYGYMLIPNVDRATFNQMIKELESSLIENNETLQSVYDAKQGVWGIVKYDDSVSTISNQFQVLKRGVYTIRKEGDEYKIAYYNPETQESAPDQEVFKKLEQAAQPQVQNSKEKEKSEEEKNHSDQKNLPQTGEGQSILASLGFLLLGAFYLFRRGKNN

SEQ ID NO: 4 - DNA, 2850 bp, Streptococcus pneumoniae
  DNA Sequence encoding Wilde Type bacterial hyaluronidase sequence
atggttcctattgaagctaagaaaaagtataaactgcgtttcaagattaaaacagataataaagtcgggattgccaaagttcgtatcattgaggaaagtggtaaggacaagcgattgtggaattctgcaacgacgtcaggaacaaaggactggcagaccattgaagcagactatagcccgactttagatgttgataaaatcaagctggagttattctatgaaacaggaactgggactgtttcctttaaggatattgagctggtagaggtagcagaccagccttctgaggattctcaaacagataaacaacttgaggaaaagattgatttaccaattggaaaaaaacatgtttttcctcttgcggactatacttataaggtagaaaatcctgacgttgcttcagtcaaaaatggaattttagaacctcttaaggaagggacaaccaatgtcattgtcagtaaagatggcaaggaagtgaaaaagattcctttgaagattctagcctctgttaaggatacatacacagaccgtttggatgactggaatggcatcatcgctgggaatcaatactatgattctaaaaatgaccagatggccaaattaaaccaggaattggaaggaaaggtagctgatagcctatccagtatttcaagtcaggcggaccgcatctatttgtgggaaaaattttcaaattataaaacgtctgcaaatctgactgccacttatcggaaattggaggagatggccaagcaagtgaccaatccttcttctcgttattatcaagatgaaactgtcgttcgaacagtcagggattccatggaatggatgcataaacatgtctacaatagtgaaaagagcattgttgggaactggtgggattatgaaatcggtacacctcgtgccatcaacaataccttgtctctgatgaaagaatacttctctgatgaggaaattaaaaaatatacagatgtgattgaaaaatttgtaccagatcccgaacatttccgaaagacgactgataacccattcaaggctctaggtggaaacttagttgatatgggaagggtaaaagtaatagctggtttactgcgtaaggatgatcaagaaatttcttctaccattcgctcgattgagcaagtgttcaagttggtagaccaaggtgaaggtttttatcaagatggatcctatatcgaccacaccaatgttgcctatacgggtgcttatgggaatgttttgattgatggcctgtctcaactgttgccagtcattcaaaagaccaagaatccaatcgataaagataaaatgcaaaccatgtaccactggattgataaatcgtttgctcctttgctggtgaatggagagctgatggatatgagtcgtggacgctcgatcagtcgtgcaaatagcgaggggcacgtggccgcagtagaagtactaagagggattcaccgaatagcggatatgtctgaaggagaaaccaaacaacgtttgcagagtcttgtgaagaccattgttcaatcggatagttattatgatgtctttaagaatttgaagacttataaggatatcagtttgatgcaatccttgttaagtgatgcaggagtcgcaagtgttccaagaacaagttacctatctgcctttaacaagatggataaaacagccatgtacaatgcagagaaagggtttggatttggcttgtcactcttttccagtcgtaccttgaattacgaacacatgaacaaggaaaataaacgtggttggtatacgagtgatgggatgttctatctttacaatggcgatttgagtcactatagcgatggctactggccaacagttaatccatataagatgcctggtacaacagagacggatgctaagagagcggatagcgatacaggtaaagttttaccgtctgctttcgttggaacgagcaaactagatgatgccaatgcgacagcaaccatggatttcaccaactggaatcaaacattgactgctcataagagctggtttatgctaaaggataagattgcctttttaggaagcaatatccaaaacacttcaacagatactgctgcaactacaattgaccagagaaaactggaatcaagtaatccatataaagtctatgtcaatgataaagaagcctcccttacagaacaagaaaaggattatcctgaaacccaaagtgggtttttagaatcgtccgattcgaaaaagaatattggttactttttctttaagaagagttcaatcagtatgagtaaggctttgcaaaagggagcctggaaggatatcaatgaaggacagtcagacaaggaagttgaaaatgaatttcttacgattagtcaggctcataagcaaaatggagattcttatggctatatgctcattcctaacgtggatcgtgccaccttcaatcaaatgataaaagagttagaaagcagcctcatcgaaaataacgaaacccttcagtctgtttatgatgccaaacaaggagtttggggcattgtgaaatatgatgattctgtctctactatttccaaccaattccaagttttgaaacgtggagtctatactattcgaaaagaaggggatgaatataagattgcctactataatcctgaaacccaggaatcagctccagatcaggaagtctttaaaaagctagagcaagcagctcagccacaagtacagaattcaaaagaaaaggaaaaatctgaagaggaaaagaaccattcggatcaaaagaatctccctcagacaggagaaggtcagtcaatcttggcaagtctagggttcttgctacttggggcgttttatttattccgtagaggaaagaacaactaa

SEQ ID NO: 5 - protein, 8 aa, Artificial Sequence
  Strep Tag Amino Acid Sequence
WSHPQFEK

SEQ ID NO: 6 - DNA, 24 bp, Artificial Sequence
  DNA Sequence encoding Strep Tag Amino Acid Sequence
tggagccatccgcagtttgaaaaa

SEQ ID NO: 7 - protein, 6 aa, Artificial Sequence
  His Tag Amino Acid Sequence
HHHHHH

SEQ ID NO: 8 - DNA, 18 bp, Artificial Sequence
  DNA Sequence encoding His Tag Amino Acid Sequence
catcatcatcatcatcac